European Patent Specification EP 3 284 464 B1, published August 13, 2025. Title: Composition for Treating or Preventing Pancreatitis Comprising Naphthoquinone-Based Compounds. Applicant: NADIANBIO SO, Hong Seob KIM, Hyung-Jin SHEN, Aihua. The sequence listing filed with the application follows.

SEQUENCE LISTING (6 sequences)

SEQ ID NO: 1 - DNA, 20 bp, Artificial
  primer IL-1b_F
tctttgaagttgacggaccc

SEQ ID NO: 2 - DNA, 20 bp, Artificial
  primer IL-1b_R
tgagtgatactgcctgcctg

SEQ ID NO: 3 - DNA, 20 bp, Artificial
  primer GAPDH_F
tcccactcttccaccttcga

SEQ ID NO: 4 - DNA, 22 bp, Artificial
  primer GAPDH_R
agttgggatagggcctctcttg

SEQ ID NO: 5 - DNA, 20 bp, Artificial
  primer MCP-1_F
ggtccctgtcatgcttctgg

SEQ ID NO: 6 - DNA, 20 bp, Artificial
  primer MCP-1_R
ccttcttggggtcagcacag